European Patent Application EP 4 603 593 A1, published August 20, 2025. Title: METHOD FOR DETECTING A TARGET NUCLEIC ACID USING TWO PROBES HAVING DIFFERENT TM VALUES. Applicant: SEEGENE, INC. The sequence listing filed with the application follows.

SEQUENCE LISTING (10 sequences)

SEQ ID NO: 1 - DNA, 186 bp, synthetic construct
  source 1..186: mol_type = other DNA
agatttatacggtattacaactggtgatagcgttagattaggagatacaaatctttgagttaaagttgaaaaagacttaactacttatggtgaagaatctgtttttggtggtggaaaaaccctacgtgaaggtatgggaatgaattctactatgaagttagatgataaattaggtaatgctgaagt

SEQ ID NO: 2 - DNA, 23 bp, synthetic construct
  source 1..23: mol_type = other DNA
agatttatacggtattacaactg

SEQ ID NO: 3 - DNA, 23 bp, synthetic construct
  source 1..23: mol_type = other DNA
acttcagcattacctaatttatc

SEQ ID NO: 4 - DNA, 29 bp, synthetic construct
  source 1..29: mol_type = other DNA
ggtgaagaatctgtttttggtggtggaaa

SEQ ID NO: 5 - DNA, 21 bp, synthetic construct
  source 1..21: mol_type = other DNA
cctacgtgaaggtatgggaat

SEQ ID NO: 6 - DNA, 205 bp, synthetic construct
  source 1..205: mol_type = other DNA
ctttattaggaggaactgaaataggaaaattcacagtcacacccaaaagctctgggagcatgttcttagtctcagcagatattattgcatcaagaatggaaggcggcgttgttctagctttggtacgagaaggtgattctaagccctgcgcgattagttatggatactcatcaggcgttcctaatttatgtagtctaagaaccag

SEQ ID NO: 7 - DNA, 25 bp, synthetic construct
  source 1..25: mol_type = other DNA
ctttattaggaggaactgaaatagg

SEQ ID NO: 8 - DNA, 26 bp, synthetic construct
  source 1..26: mol_type = other DNA
ctggttcttagactacataaattagg

SEQ ID NO: 9 - DNA, 34 bp, synthetic construct
  source 1..34: mol_type = other DNA
tgcatcaagaatggaaggcggcgttgttctagct

SEQ ID NO: 10 - DNA, 29 bp, synthetic construct
  source 1..29: mol_type = other DNA
ggtacgagaaggtgattctaagccctgcg